European Patent Application EP 4 342 471 A1, published March 27, 2024. Title: 一种调节神经病变的方法. Applicant: 成都文鼎科技发展有限公司. The sequence listing filed with the application follows.

SEQUENCE LISTING (8 sequences)

SEQ ID NO: 1 - DNA, 24 bp, 人工序列(Artificial Sequence)
tcgtgcgtgacattaaggagaagc

SEQ ID NO: 2 - DNA, 23 bp, 人工序列(Artificial Sequence)
tcgttgccaatggtgatgacctg

SEQ ID NO: 3 - DNA, 24 bp, 人工序列(Artificial Sequence)
cgaatgtccaacgcaaagcagtac

SEQ ID NO: 4 - DNA, 24 bp, 人工序列(Artificial Sequence)
tgctcttcgacctcgaaacatctg

SEQ ID NO: 5 - DNA, 24 bp, 人工序列(Artificial Sequence)
cttactacagcggcaacgaggatg

SEQ ID NO: 6 - DNA, 20 bp, 人工序列(Artificial Sequence)
ccaccacccagagggcagag

SEQ ID NO: 7 - DNA, 24 bp, 人工序列(Artificial Sequence)
aatggcgtggagctgacagataac

SEQ ID NO: 8 - DNA, 20 bp, 人工序列(Artificial Sequence)
cgatgcggctgatggtgtgg